European Patent Specification EP 4 019 530 B1, published April 10, 2024. Title: Peptide having activities of skin condition improvement and uses thereof. Applicant: CAREGEN CO., LTD. The sequence listing filed with the application follows.

SEQUENCE LISTING (27 sequences)

SEQ ID NO: 1 - protein, 8 aa, Artificial Sequence
  Peptide 1
ECEELEEK

SEQ ID NO: 2 - DNA, 20 bp, Artificial Sequence
  PPAR-gamma_F
acgatctgcctgaggtctgt

SEQ ID NO: 3 - DNA, 20 bp, Artificial Sequence
  PPAR-gamma_R
catcgaggacatccaagaca

SEQ ID NO: 4 - DNA, 20 bp, Artificial Sequence
  PPAR-delta_F
ctgaagggaagggggtagag

SEQ ID NO: 5 - DNA, 19 bp, Artificial Sequence
  PPAR-delta_R
cagtctggatgctgctaca

SEQ ID NO: 6 - DNA, 20 bp, Artificial Sequence
  PGC-1alpha_F
actgagctacccttgggatg

SEQ ID NO: 7 - DNA, 20 bp, Artificial Sequence
  PGC-1alpha_R
taaggatttcggtggtgaca

SEQ ID NO: 8 - DNA, 25 bp, Artificial Sequence
  GAPDH_F
ggtgtgaacggatttggccgtattg

SEQ ID NO: 9 - DNA, 25 bp, Artificial Sequence
  GAPDH_R
ccgttgaatttgccgtgagtggagt

SEQ ID NO: 10 - DNA, 20 bp, Artificial Sequence
  Col1a1_F
caccctcaagagcctgagtc

SEQ ID NO: 11 - DNA, 20 bp, Artificial Sequence
  Col1a1_R
agacggctgagtagggaaca

SEQ ID NO: 12 - DNA, 20 bp, Artificial Sequence
  Fibronectin_F
ccaggaaccgagtacaccat

SEQ ID NO: 13 - DNA, 20 bp, Artificial Sequence
  Fibronectin_R
atacccaggttgggtgatga

SEQ ID NO: 14 - DNA, 20 bp, Artificial Sequence
  Elastin_F
ggacccctgactcgcgacct

SEQ ID NO: 15 - DNA, 20 bp, Artificial Sequence
  Elastin_R
ggggaggtgggactgcccaa

SEQ ID NO: 16 - DNA, 20 bp, Artificial Sequence
  SIRT1_F
tcagtggctggaacagtgag

SEQ ID NO: 17 - DNA, 20 bp, Artificial Sequence
  SIRT1_R
tctggcatgtcccactatca

SEQ ID NO: 18 - DNA, 20 bp, Artificial Sequence
  AQP3_F
ccttcttgggtgctggaata

SEQ ID NO: 19 - DNA, 20 bp, Artificial Sequence
  AQP3_R
acacgataagggaggctctg

SEQ ID NO: 20 - DNA, 21 bp, Artificial Sequence
  TNF-alpha_F
cgtcagccgattrtgctatct

SEQ ID NO: 21 - DNA, 20 bp, Artificial Sequence
  TNF-alpha_R
cggactccgcaaagtctaag

SEQ ID NO: 22 - DNA, 21 bp, Artificial Sequence
  COX-2_F
atcattcaccaggcaaattgc

SEQ ID NO: 23 - DNA, 21 bp, Artificial Sequence
  COX-2_R
ggcttcagcataaagcgtttg

SEQ ID NO: 24 - DNA, 20 bp, Artificial Sequence
  IL-1beta_F
ttcgacacatgggataacga

SEQ ID NO: 25 - DNA, 20 bp, Artificial Sequence
  IL-1beta_R
tctttcaacacgcaggacag

SEQ ID NO: 26 - DNA, 20 bp, Artificial Sequence
  IL-6_F
aaagaggcactgccagaaaa

SEQ ID NO: 27 - DNA, 20 bp, Artificial Sequence
  IL-6_R
atctgaggtgcccatgctac